European Patent Application EP 4 567 045 A1, published June 11, 2025. Title: ANTI-DDR2 NANO-ANTIBODY AND USE THEREOF. Applicant: Fibro-Biomed Technology (Guangzhou) Company, Ltd. The sequence listing filed with the application follows.

SEQUENCE LISTING (27 sequences)

SEQ ID NO: 1 - protein, 8 aa, synthetic construct
GRIFSINV

SEQ ID NO: 2 - protein, 8 aa, synthetic construct
INTRGGST

SEQ ID NO: 3 - protein, 17 aa, synthetic construct
AASRKGYPSTRSDPYDY

SEQ ID NO: 4 - protein, 124 aa, synthetic construct
EVQLVESGGGLVQPGGSLRLSCAASGRIFSINVMGWFRQAPGKGRELVAAINTRGGSTYYPDSVEGRFTISRDNAKRMVYLQMNSLRAEDTAVYYCAASRKGYPSTRSDPYDYWGQGTQVTVSS

SEQ ID NO: 5 - protein, 8 aa, synthetic construct
GITLSLYI

SEQ ID NO: 6 - protein, 8 aa, synthetic construct
ISRTGGST

SEQ ID NO: 7 - protein, 14 aa, synthetic construct
AADFYGNATLGYNY

SEQ ID NO: 8 - protein, 121 aa, synthetic construct
EVQLVESGGGLVQPGGSLRLSCAASGITLSLYIMGWFRQAPGKGRELVAAISRTGGSTYYPDSVEGRFTISRDNAKRMVYLQMNSLRAEDTAVYYCAADFYGNATLGYNYWGQGTQVTVSS

SEQ ID NO: 9 - protein, 8 aa, synthetic construct
GYILSPNV

SEQ ID NO: 10 - protein, 8 aa, synthetic construct
ISWGDGRT

SEQ ID NO: 11 - protein, 17 aa, synthetic construct
AASRKGYPSTRSDPYNY

SEQ ID NO: 12 - protein, 124 aa, synthetic construct
EVQLVESGGGLVQPGGSLRLSCAASGYILSPNVMGWFRQAPGKGRELVAAISWGDGRTYYPDSVEGRFTISRDNAKRMVYLQMNSLRAEDTAVYYCAASRKGYPSTRSDPYNYWGQGTQVTVSS

SEQ ID NO: 13 - protein, 8 aa, synthetic construct
GYIFSIYA

SEQ ID NO: 14 - protein, 8 aa, synthetic construct
ISWGDGST

SEQ ID NO: 15 - protein, 17 aa, synthetic construct
AAAIKGRGVVTQLGYNY

SEQ ID NO: 16 - protein, 124 aa, synthetic construct
EVQLVESGGGLVQPGGSLRLSCAASGYIFSIYAMGWFRQAPGKGRELVARISWGDGSTWYPDSVEGRFTISRDNAKRMVYLQMNSLRAEDTAVYYCAAAIKGRGVVTQLGYNYWGQGTQVTVSS

SEQ ID NO: 17 - protein, 8 aa, synthetic construct
GDTFSYYV

SEQ ID NO: 18 - protein, 8 aa, synthetic construct
ISRTGGST

SEQ ID NO: 19 - protein, 14 aa, synthetic construct
AADPYISGTLGYNY

SEQ ID NO: 20 - protein, 121 aa, synthetic construct
EVQLVESGGGLVQPGGSLRLSCAASGDTFSYYVMGWFRQAPGKGRELVAAISRTGGSTYYPDSVEGRFTISRDNAKRMVYLQMNSLRAEDTAVYYCAADPYISGTLGYNYWGQGTQVTVSS

SEQ ID NO: 21 - DNA, 372 bp, synthetic construct
  source 1..372: mol_type = other DNA
gaggtgcagctggtggagagcggtggtggtctcgtgcagcccggcggtagtctgcgcctcagctgtgccgccagcggtcgcatctttagcatcaatgtgatgggctggtttcgccaagcccccggcaaaggtcgcgaactggtggccgccattaacacccgcggtggcagcacctattacccagatagcgtggaaggccgcttcaccatcagccgcgataacgccaagcgcatggtgtatctgcagatgaacagtctgcgcgccgaggacaccgccgtgtattattgtgccgccagccgcaaaggctatccaagcacccgcagcgatccatacgattactggggccaaggcacccaagtgaccgtgagcagc

SEQ ID NO: 22 - DNA, 363 bp, synthetic construct
  source 1..363: mol_type = other DNA
gaggtgcagctggtggagagcggtggtggtctcgtgcagcccggcggtagtctgcgcctcagctgtgccgccagcggtatcacccttagcctgtatatcatgggctggtttcgccaagcccccggcaaaggtcgcgaactggtggccgccatttcccgcacgggcggtagcacctactacccagatagcgtggaaggccgcttcaccatcagccgcgataacgccaagcgcatggtgtatctgcagatgaacagtctgcgcgccgaggacaccgccgtgtattattgtgccgccgatttttatggcaacgccaccctgggctacaattactggggccaaggcacccaagtgaccgtgagcagc

SEQ ID NO: 23 - DNA, 372 bp, synthetic construct
  source 1..372: mol_type = other DNA
gaggtgcagctggtggagagcggtggtggtctcgtgcagcccggcggtagtctgcgcctcagctgtgccgccagcggttatatccttagcccaaatgtgatgggctggtttcgccaagcccccggcaaaggtcgcgaactggtggccgccattagctggggcgatggccgcacctattacccagatagcgtggaaggccgcttcaccatcagccgcgataacgccaagcgcatggtgtatctgcagatgaacagtctgcgcgccgaggacaccgccgtgtattattgtgccgccagccgcaaaggctatccaagcacccgcagcgatccatacaattactggggccaaggcacccaagtgaccgtgagcagc

SEQ ID NO: 24 - DNA, 372 bp, synthetic construct
  source 1..372: mol_type = other DNA
gaggtgcagctggtggagagcggtggtggtctcgtgcagcccggcggtagtctgcgcctcagctgtgccgccagcggttatatctttagcatctatgccatgggctggtttcgccaagcccccggcaaaggtcgcgaactggtggcccgcattagctggggcgatggcagcacctggtacccagatagcgtggaaggccgcttcaccatcagccgcgataacgccaagcgcatggtgtatctgcagatgaacagtctgcgcgccgaggacaccgccgtgtattattgtgccgccgccatcaaaggccgcggcgtggtgacccagctgggctacaattactggggccaaggcacccaagtgaccgtgagcagc

SEQ ID NO: 25 - DNA, 363 bp, synthetic construct
  source 1..363: mol_type = other DNA
gaggtgcagctggtggagagcggtggtggtctcgtgcagcccggcggtagtctgcgcctcagctgtgccgccagcggtgatacctttagctattatgtgatgggctggtttcgccaagcccccggcaaaggtcgcgaactggtggccgccatttcccgcacgggcggtagcacctactacccagatagcgtggaaggccgcttcaccatcagccgcgataacgccaagcgcatggtgtatctgcagatgaacagtctgcgcgccgaggacaccgccgtgtattattgtgccgccgatccatatatcagcggcaccctgggctacaattactggggccaaggcacccaagtgaccgtgagcagc

SEQ ID NO: 26 - protein, 4 aa, synthetic construct
GGGS

SEQ ID NO: 27 - protein, 12 aa, synthetic construct
GGGSGGGSGGGS